European Patent Application EP 4 556 573 A2, published May 21, 2025. Title: METHODS FOR PERFORMING SPATIAL PROFILING OF BIOLOGICAL MOLECULES. Applicant: Centrillion Technology Holdings Corporation. Application EP. The sequence listing filed with the application follows.

SEQUENCE LISTING (36 sequences)

SEQ ID NO: 1 - DNA, 22 bp, synthetic construct
  misc_feature 1..22: note = Description of Artificial Sequence: Synthetic oligonucleotide
  source 1..22: mol_type = other DNA
agcgcttagcctagagctctag

SEQ ID NO: 2 - DNA, 23 bp, synthetic construct
  misc_feature 1..23: note = Description of Artificial Sequence: Synthetic oligonucleotide
  source 1..23: mol_type = other DNA
gcgcttagcttagagctctattg

SEQ ID NO: 3 - DNA, 19 bp, synthetic construct
  misc_feature 1..19: note = Description of Artificial Sequence: Synthetic oligonucleotide
  source 1..19: mol_type = other DNA
agatgtgtataagagacag

SEQ ID NO: 4 - DNA, 19 bp, synthetic construct
  misc_feature 1..19: note = Description of Artificial Sequence: Synthetic oligonucleotide
  source 1..19: mol_type = other DNA
ctgtctcttatacacatct

SEQ ID NO: 5 - DNA, 46 bp, synthetic construct
  misc_feature 1..46: note = Description of Artificial Sequence: Synthetic oligonucleotide
  source 1..46: mol_type = other DNA
gactcgtaatacgactcactatagggacacgacgctcttccgatct

SEQ ID NO: 6 - DNA, 100 bp, synthetic construct
  misc_feature 1..100: note = Description of Artificial Sequence: Synthetic polynucleotide
  variation 47..76: note = a, c, t, or g
  variation 100: note = a, c, t, g, unknown or other
  source 1..100: mol_type = other DNA
gactcgtaatacgactcactatagggacacgacgctcttccgatctnnnnnnnnnnnnnnnnnnnnnnnnnnnnnngattttttttttttttttttttvn

SEQ ID NO: 7 - DNA, 35 bp, synthetic construct
  misc_feature 1..35: note = Description of Artificial Sequence: Synthetic oligonucleotide
  source 1..35: mol_type = other DNA
agatcggaagagcacacgtctgaactccagtcacc

SEQ ID NO: 8 - DNA, 34 bp, synthetic construct
  misc_feature 1..34: note = Description of Artificial Sequence: Synthetic primer
  source 1..34: mol_type = other DNA
gtgactggagttcagacgtgtgctcttccgatct

SEQ ID NO: 9 - DNA, 58 bp, synthetic construct
  misc_feature 1..58: note = Description of Artificial Sequence: Synthetic oligonucleotide
  source 1..58: mol_type = other DNA
aatgatacggcgaccaccgagatctacactctttccctacacgacgctcttccgatct

SEQ ID NO: 10 - DNA, 58 bp, synthetic construct
  misc_feature 1..58: note = Description of Artificial Sequence: Synthetic oligonucleotide
  source 1..58: mol_type = other DNA
caagcagaagacggcatacgagatgtgactggagttcagacgtgtgctcttccgatct

SEQ ID NO: 11 - DNA, 52 bp, synthetic construct
  misc_feature 1..52: note = Description of Artificial Sequence: Synthetic oligonucleotide
  variation 24..25: note = a, c, t, g, unknown or other
  variation 28..29: note = a, c, t, g, unknown or other
  variation 52: note = a, c, t, g, unknown or other
  source 1..52: mol_type = other DNA
agacgtgtgctcttccgatctwsnnwsnnvttttttttttttttttttttvn

SEQ ID NO: 12 - DNA, 39 bp, synthetic construct
  misc_feature 1..39: note = Description of Artificial Sequence: Synthetic oligonucleotide
  misc_feature 1..39: note = Description of Combined DNA/RNA Molecule: Synthetic oligonucleotide
  source 1..39: mol_type = other DNA
  misc_feature 1..36: note = DNA
  misc_feature 37..39: note = RNA
cgcacactctttccctacacgacgctcttccgatctggg

SEQ ID NO: 13 - DNA, 83 bp, synthetic construct
  misc_feature 1..83: note = Description of Artificial Sequence: Synthetic oligonucleotide
  variation 34..63: note = a, c, t, or g
  source 1..83: mol_type = other DNA
agatcggaagagcgtcgtgtagggaaagagtgtnnnnnnnnnnnnnnnnnnnnnnnnnnnnnnaagagacgcgctgaccctga

SEQ ID NO: 14 - DNA, 45 bp, synthetic construct
  misc_feature 1..45: note = Description of Artificial Sequence: Synthetic oligonucleotide
  source 1..45: mol_type = other DNA
aatgatacggcgaccaccgagatcttcagggtcagcgcgtctctt

SEQ ID NO: 15 - DNA, 21 bp, synthetic construct
  misc_feature 1..21: note = Description of Artificial Sequence: Synthetic oligonucleotide
  source 1..21: mol_type = other DNA
gcgcttagcctagagctctag

SEQ ID NO: 16 - DNA, 21 bp, synthetic construct
  misc_feature 1..21: note = Description of Artificial Sequence: Synthetic oligonucleotide
  source 1..21: mol_type = other DNA
gcgcttagcttagagctctag

SEQ ID NO: 17 - DNA, 22 bp, synthetic construct
  misc_feature 1..22: note = Description of Artificial Sequence: Synthetic oligonucleotide
  source 1..22: mol_type = other DNA
gcgcttagcttagagctctatg

SEQ ID NO: 18 - DNA, 12 bp, synthetic construct
  misc_feature 1..12: note = Description of Artificial Sequence: Synthetic oligonucleotide
  source 1..12: mol_type = other DNA
accgatctagca

SEQ ID NO: 19 - DNA, 13 bp, synthetic construct
  misc_feature 1..13: note = Description of Artificial Sequence: Synthetic oligonucleotide
  source 1..13: mol_type = other DNA
gaccgatctagca

SEQ ID NO: 20 - DNA, 12 bp, synthetic construct
  misc_feature 1..12: note = Description of Artificial Sequence: Synthetic oligonucleotide
  source 1..12: mol_type = other DNA
gacgatctagca

SEQ ID NO: 21 - DNA, 13 bp, synthetic construct
  misc_feature 1..13: note = Description of Artificial Sequence: Synthetic oligonucleotide
  source 1..13: mol_type = other DNA
gacgcatctagca

SEQ ID NO: 22 - DNA, 27 bp, synthetic construct
  misc_feature 1..27: note = Description of Artificial Sequence: Synthetic oligonucleotide
  source 1..27: mol_type = other DNA
gacgatctagcattgaccgatctagca

SEQ ID NO: 23 - DNA, 26 bp, synthetic construct
  misc_feature 1..26: note = Description of Artificial Sequence: Synthetic oligonucleotide
  source 1..26: mol_type = other DNA
gacgatctagcattaccgatctagca

SEQ ID NO: 24 - DNA, 28 bp, synthetic construct
  misc_feature 1..28: note = Description of Artificial Sequence: Synthetic oligonucleotide
  source 1..28: mol_type = other DNA
gacgcatctagcattgaccgatctagca

SEQ ID NO: 25 - DNA, 27 bp, synthetic construct
  misc_feature 1..27: note = Description of Artificial Sequence: Synthetic oligonucleotide
  source 1..27: mol_type = other DNA
gacgcatctagcattaccgatctagca

SEQ ID NO: 26 - DNA, 35 bp, synthetic construct
  misc_feature 1..35: note = Description of Artificial Sequence: Synthetic oligonucleotide
  variation 3..14: note = a, c, t, g, unknown or other
  variation 22..33: note = a, c, t, g, unknown or other
  source 1..35: mol_type = other DNA
hhnnnnnnnnnnnnhhggghhnnnnnnnnnnnnhh

SEQ ID NO: 27 - DNA, 16 bp, synthetic construct
  misc_feature 1..16: note = Description of Artificial Sequence: Synthetic oligonucleotide
  source 1..16: mol_type = other DNA
caagttcctacagcta

SEQ ID NO: 28 - DNA, 16 bp, synthetic construct
  misc_feature 1..16: note = Description of Artificial Sequence: Synthetic oligonucleotide
  source 1..16: mol_type = other DNA
agtccatgcccatccg

SEQ ID NO: 29 - DNA, 16 bp, synthetic construct
  misc_feature 1..16: note = Description of Artificial Sequence: Synthetic oligonucleotide
  source 1..16: mol_type = other DNA
aatcggacttcagcct

SEQ ID NO: 30 - DNA, 16 bp, synthetic construct
  misc_feature 1..16: note = Description of Artificial Sequence: Synthetic oligonucleotide
  source 1..16: mol_type = other DNA
gacctaagccatcaga

SEQ ID NO: 31 - DNA, 16 bp, synthetic construct
  misc_feature 1..16: note = Description of Artificial Sequence: Synthetic oligonucleotide
  source 1..16: mol_type = other DNA
aatcctagcatccagc

SEQ ID NO: 32 - DNA, 16 bp, synthetic construct
  misc_feature 1..16: note = Description of Artificial Sequence: Synthetic oligonucleotide
  source 1..16: mol_type = other DNA
accgttacatcaacag

SEQ ID NO: 33 - DNA, 16 bp, synthetic construct
  misc_feature 1..16: note = Description of Artificial Sequence: Synthetic oligonucleotide
  source 1..16: mol_type = other DNA
attcgataacgaccat

SEQ ID NO: 34 - DNA, 16 bp, synthetic construct
  misc_feature 1..16: note = Description of Artificial Sequence: Synthetic oligonucleotide
  source 1..16: mol_type = other DNA
catgccattgacgatt

SEQ ID NO: 35 - DNA, 20 bp, synthetic construct
  misc_feature 1..20: note = Description of Artificial Sequence: Synthetic oligonucleotide
  source 1..20: mol_type = other DNA
aaaaaaaaaaaaaaaaaaaa

SEQ ID NO: 36 - DNA, 23 bp, synthetic construct
  misc_feature 1..23: note = Description of Artificial Sequence: Synthetic oligonucleotide
  source 1..23: mol_type = other DNA
ttttttttttttttttttttttt